European Patent Specification EP 3 802 788 B1, published July 2, 2025. Title: SYSTEMS AND METHODS FOR GENETIC MANIPULATION OF AKKERMANSIA SPECIES. Applicant: Valdivia, Raphael Malkus, Per Davey, Lauren. The sequence listing filed with the application follows.

SEQUENCE LISTING (47 sequences)

SEQ ID NO: 1 - DNA, 4476 bp, Artificial Sequence
  pSAM_Akk transposon vector
  bla_complement (1)..(861)
  KpnI (1072)..(1077)
  transposon (1078)..(2267)
  MmeI IR_L (1078)..(1106)
  inverted repeat left (1080)..(1107)
  MmeI_complement (1084)..(1089)
  BioSamA primer binding site (1102)..(1127)
  AscI (1127)..(1134)
  XhoI (1135)..(1140)
  MfeI (1141)..(1145)
  cat (1148)..(1960)
  terminator (1991)..(2034)
  terminator (2166)..(2193)
  BioSamA primer binding site (2218)..(2243)
  P7 (2219)..(2238)
  inverted repeat right (2238)..(2265)
  MmeI IR_R (2239)..(2267)
  Bt1311 promoter (2274)..(2570)
  Himar codon optimized (2571)..(3628)
  RP4-OriT-OriR6K (3629)..(4428)
ttaccaatgcttaatcagtgaggcacctatctcagcgatctgtctatttcgttcatccatagttgcctgactccccgtcgtgtagataactacgatacgggagggcttaccatctggccccagtgctgcaatgataccgcgagacccacgctcaccggctccagatttatcagcaataaaccagccagccggaagggccgagcgcagaagtggtcctgcaactttatccgcctccatccagtctattaattgttgccgggaagctagagtaagtagttcgccagttaatagtttgcgcaacgttgttgccattgctacaggcatcgtggtgtcacgctcgtcgtttggtatggcttcattcagctccggttcccaacgatcaaggcgagttacatgatcccccatgttgtgcaaaaaagcggttagctccttcggtcctccgatcgttgtcagaagtaagttggccgcagtgttatcactcatggttatggcagcactgcataattctcttactgtcatgccatccgtaagatgcttttctgtgactggtgagtactcaaccaagtcattctgagaatagtgtatgcggcgaccgagttgctcttgcccggcgtcaatacgggataataccgcgccacatagcagaactttaaaagtgctcatcattggaaaacgttcttcggggcgaaaactctcaaggatcttaccgctgttgagatccagttcgatgtaacccactcgtgcacccaactgatcttcagcatcttttactttcaccagcgtttctgggtgagcaaaaacaggaaggcaaaatgccgcaaaaaagggaataagggcgacacggaaatgttgaatactcatactcttcctttttcaatattattgaagcatttatcagggttattgtctcatgagcggatacatatttgaatgtatttagaaaaataaacaaataggggttccgcgcacatttccccgaaaagtgccacctgacgtctaagaaaccattattatcatgacattaacctataaaaataggcgtatcacgaggccctttcgtcacgcgtcctcggtacctaacaggttggatgataagtccccggtcttcgtatgccgtcttctgcttggcgcgccctcgagcaattgcgctcgtaagaggttccaactttcaccataatgaaataagatcactaccgggcgtattttttgagttatcgagattttcaggagctaaggaagctaaaatggagaaaaaaatcactggatataccaccgttgatatatcccaatggcatcgtaaagaacattttgaggcatttcagtcagttgctcaatgtacctataaccagaccgttcagctggatattacggcctttttaaagaccgtaaagaaaaataagcacaagttttatccggcctttattcacattcttgcccgcctgatgaatgctcatccggaattccgtatggcaatgaaagacggtgagctggtgatatgggatagtgttcacccttgttacaccgttttccatgagcaaactgaaacgttttcatcgctctggagtgaataccacgacgatttccggcagtttctacacatatattcgcaagatgtggcgtgttacggtgaaaacctggcctatttccctaaagggtttattgagaatatgtttttcgtctcagccaatccctgggtgagtttcaccagttttgatttaaacgtggccaatatggacaacttcttcgcccccgttttcaccatgggcaaatattatacgcaaggcgacaaggtgctgatgccgctggcgattcaggttcatcatgccgtttgtgatggcttccatgtcggcagaatgcttaatgaattacaacagtactgcgatgagtggcagggcggggcgtaatttttttaaggcagttattggtgcccttaaacgcctggtgctacgcctgaataagtatgcgagagtagggaactgccaggcatcaaataaaacgaaaggctcagtcgaaagactgggcctttcgttttatctgttgtttgtcggtgaacgctctcctgagtaggacaaatccgccgggagcggatttgaacgttgcgaagcaacggcccggagggtggcgggcaggacgcccgccataaactgccaggcatcaaattaagcagaaggccatcctgacggatggcctttttgcgtttctacctgcagggcgcgccaagcagaagacggcatacgaagaccggggacttatcatccaacctgttaggatcctgatctggaagaagcaatgaaagctgctgttaagtctccgaatcaggtattgttcctgacaggtgtattcccatccggtaaacgcggatactttgcagttgatctgactcaggaataaattataaattaaggtaagaagattgtaggataagctaatgaaatagaaaaaggatgccgtcacacaacttgtcggcattcttttttgttttattagttgaaaatatagtgaaaaagttgcctaaatatgtatgttaacaaattatttgtcgtaactttgcactccaaatctgtttttaacatatggaaaaaaaggaatttagggttttgataaaatactgttttctgaagggaaaaaatacagtggaagcaaaaacttggcttgataatgagtttccggactctgccccagggaaatcaacaataattgattggtatgcaaaattcaagaggggtgaaatgagcacggaggacggtgaacgcagtggacgcccgaaagaggtggttaccgacgaaaacatcaaaaaaatccacaaaatgattttgaatgacaggaaaatgaagttgatcgagatagcagaggccttaaagatatcaaaggaaagggttggtcatatcattcatcaatatttggatatgcggaagctctgtgcgaaatgggtgccgcgcgagctcacatttgaccaaaaacaacggagggttgatgattcaaagcggtgtttgcagctgttaactaggaatacacccgagtttttcaggcggtatgtgacaatggatgaaacatggctccatcactacactcctgagtccaatcggcagtcggctgagtggacagcgaccggtgaaccgtcaccgaagaggggaaagactcaaaagtccgctggcaaagtaatggcctcagttttttgggatgcgcatggaataatttttatcgattatcttgagaagggaaaaaccatcaacagtgactattatatggcgttattggagaggttgaaggtcgaaatcgcggcaaaacggccccacatgaagaagaaaaaagtgttgttccaccaagacaacgcaccgtgccacaagtcattgagaacgatggcaaaaattcatgaattgggcttcgaattgcttccccacccgccgtattcaccagatctggcccccagcgactttttcttgttctcagacctcaaaaggatgctcgcagggaaaaaatttggctgcaatgaagaggtgatcgccgaaactgaggcctattttgaggcaaaaccgaaggagtactaccaaaatggtatcaaaaaattggaaggtaggtataataggtgtatcgctcttgaagggaactatgttgaataagcggccgccaccgcggtggaggggaattcccatgtcagccgttaagtgttcctgtgtcactcaaaattgctttgagaggctctaagggcttctcagtgcgttacatccctggcttgttgtccacaaccgttaaaccttaaaagctttaaaagccttatatattcttttttttcttataaaacttaaaaccttagaggctatttaagttgctgatttatattaattttattgttcaaacatgagagcttagtacgtgaaacatgagagcttagtacgttagccatgagagcttagtacgttagccatgagggtttagttcgttaaacatgagagcttagtacgttaaacatgagagcttagtacgtgaaacatgagagcttagtacgtactatcaacaggttgaactgctgatcttcagatcctctacgccggacgcatcgtggccggatcaattccgttttccgctgcataaccctgcttcggggtcattatagcgattttttcggtatatccatcctttttcgcacgatatacaggattttgccaaagggttcgtgtagactttccttggtgtatccaacggcgtcagccgggcaggataggtgaagtaggcccacccgcgagcgggtgttccttcttcactgtcccttattcgcacctggcggtgctcaacgggaatcctgctctgcgaggctggccggctaccgccggcgtaacagatgagggcaagcggatggctgatgaaaccaagccaaccaggaagggcagcccacctatcacggaattgatccccctcgaattgacgcgtaagggcagcccacctatcacggaattgatccccctcgaattgacgcgt

SEQ ID NO: 2 - DNA, 927 bp, Akkermansia muciniphila
atgaagattctcgtaaccggcggcgccggattcatcggttcccacattgtggaacactatcaggataaggcggaggaaatccgtgtgctggacaacctgcgcacgggctatctcaagaacctggaagggctcaggcacacgttcatcgaaggttccatctgcgaccgggagctggtgcgccaggcggtgcagggagtggactatattttccacatggccgcgctcgtctccgtgccggaatccatgagcaagatcagcgaatgcatcgacatcaacgtcaacggtttgctgaacgtgctggaggaagcttccgccgccggagtcaaaaaaatcgtgctggcgtcttccgccgccatttacggagacaatcccacggtgcccaaactggaaaccatgtacccggaacccaagagtccctatgccattaccaagctggatggggaatactacctcaacatgttccgggcggaaggaaaaattaatacggcagccgtgcgcttcttcaatgtcttcggcccccggcaggaccccaagggcgcctatgccgcagccgtgcccattttcattgaaaaagctgtcaaaggagaagacatcaccgtgtatggggacggctcccagacgcgcgatttcatttatgtgaaagacattgtaggagccctcacctttgtggcggaacacccggaagtcaccggcgtgttcaatgccggttacggcggccagatcaccattgaagagctggcgcagaacatcatcaaggctgccgggtcttcctccaaggtgcttcatgccccggaacgtccgggagacgtcaagcattcccgcgcctgtgcggacaagctccgcaatgccggatggcagcccaggcatactttgccggaaggcctggcgacgacgctggaatacttcaagggcattctgggcaggtaa

SEQ ID NO: 3 - DNA, 1290 bp, Akkermansia muciniphila
atgttcccgtttcctcctgttgtccgttctttcctgttttccctgtttgaaagggcatggctgagggctgcgttgtgcttctgcctctgtacggcggtatgcgcctcctgctccgtggacaggcacatggaaaaaaaggcgggggaattgatggccaggatggatgccgttcccgattggcggcagctgccgcggaaggaaatctcatggcaccaggccctggcgatgatgatggagcggaacattgacttgaaaaaatcggagcagtccctcaagacgacgaaacgttccgtcgttaatgtttttacccagattatccccggagtcaatctggactggatgctgaccaaggaattgagcgacctggccagggtgacggccagcgatgtggaatacaatacgaacattctgttcaacatgccgtccctcacccagatcccgtttgattattattccgccaaggcggctgtttatacggcggaaaagacgctggagatgaaaaaaagggagctggtggccagattgtaccagcaggtgctttcctaccggaacgcgcagatcagctacaataaccagctgagctccctgccttatgacgatgatggcgtccagaaaaagaagctggacctggaacgggagcggaatttgaatgagatttcccaggggtttgccgtgttgctggggaatatggacgcccggtggctggtgaaccctgaaacgatgcccaggctggactggggcaggtacagggcggcgtcccggcagctggatctgctggtggtgacgatggtggccatggagctggaagcttcccgcctccaggtgctgaatgccaaactgaagttcttcccgtccgtggatattaatttttacagcccaaccctgttttccagcacgggcgggacgtacggcggtttttttgcgggagcgggcgatatgaaggtgaacatgagcctgcgggaagaactggatacgcgcctgacatcctggttccagtataagtcggccaaagaaagccacgaactgctgcagcgcgaagtggtgatggaactgcagcggcggcgtatcaagatagccgcgttgctggagagccgcaggaggtttgagctctggcagggggtgctgatgaaggaaatcgcgttcaaggagtccagattatccgtttccggagatgaatatctggaacagaggaaggatatcaggaaaatgtatgctgacctggataatgaagcttccaagaatgcggaggtggaagcggccctcatcatggaatatggctggctgaagtaa

SEQ ID NO: 4 - DNA, 759 bp, Akkermansia muciniphila
atgaaagtatcttttgcaacacaccagttacgcagggggtttaccctgattgaactcttggttgtcattgccattatcgccctgctggcttccgtggcctatggtcctatcctgaaccagatcaacaaaggcgaccagatgcaggccctgaccaacatgaagaacgtgggcgtagcgatgaacgagttcaaatccaacagcaaactgggcaatttccccgatgacatcactgccgaccgcgttgttgcccagcataattatatgagcggcctgggcgcacttcagggcgatacttccaatgactatttccgtcagcttctgggcaatgagtctgtttccgaaagcaacttttacgccaaagttcagactccttccggcggttccaccgttactcccaacggtgaaatttacgacggtcaggccctgacccccggtgaagtgggtatttcctacgtcatgcgcaagggtgacaataacaagaaagtgggtattggaagttccgtgggggaatatcccctgatggtcacttccgtgcttcctggtgaagacggcagcaccgttgtggctggcaatgccgtgcgttttgacccggaaagcttccgcggcaaggttctgattttcacgactgcccagagtgccaagaccctggaactggacgacaacgacaaccttcaggataccttcattcccaagagaaggggcaaggacatcagcgaccagttcctgatcctcacgcctgatttcagcggccaggagtaa

SEQ ID NO: 5 - DNA, 1023 bp, Akkermansia muciniphila
atggtattggccggactgtcctccctggttccgtccatggcccagaatgcccagaatccccagcgcctgcgcgccagagttgccgcaccgaccatcaagaatggccgtccgacggatatctacattctttcctccaatggacccacggtccagtttgtggagagcagggaatcccaggaagtccttcagcagatggccagcgccttcaagacgctgtatatttttgaaacggacgactttgtggatgccaaggtggctatggaaaaccggaagtaccaggaagcccgcaacaaattccacgctctggtgaataagtatgcctcaacgctttccatcaaggacagcctgtccgcccgggcggccgtctatgaactggagtgcgccatgcgcatgatggattgggctggagtcaaagggttggcggccaagtttcccgtcagaggggccaatttgtccccttccgcccagaatgacctggaggtggcaaaaatcatggccttgattccagataaggactggaacggcgtgaaaagccgtgccggttctttcctggcaaccaaaaagaatgccacccgcctccagcaggcgcggatgaaatatgccctgggtgcggccgccatggtggcccaggattggaacaaggcgctggattattttgcggaagccctggttttgttgcatggttccgatgaagaactggcgtctgcctgcgtggcccgctccctggatgcctacctgcgcatgccggatgttgtcaaattctttgagaatcccgtcgtctcatctgccgtggaatccaggaagaataatcccgaagctgtgattccggattcacggctgaagtcccgtcccgttcctgtcaaggaagcggctgccctgtaccgtttgcatgaactgatgttcccggacaggaagctgccggccaagtatgacggttttgcggtttcctacaagcatccggccgctgttgctcccgccaaggctcctgaccaggctcccgcacagccgcagaataagcagtaa

SEQ ID NO: 6 - DNA, 3234 bp, Akkermansia muciniphila
atgatcaaatcaaactatactactgcactggctgcaggcctggtttccgtgctgagtatcggggcggttcttccatccggcgcccagcatggcccgcgcgattaccagcgcacggccctgacggccattaaggaagggaagtggcaggaagccctggatgccgtggatcgctgcatccgcgtttatgaaccccgtatcaagatgctggggctggatgacggcttcggctggttctattaccagaagggcgtctgtctggcccagctgaaaaattacaaggaggctgtggaagcgttcaaggcttgttacaccaagtttccgagcgctaaaaaccagctcgtgaaaatggccctgttccgggaaggggaaaactactgccgtcttggggattttgccaagggtgcggagctgctggaaaaattcctgaaagaataccgcagcgatcctgtcgccagaaacgtcaatgctggcgaagtgcaggggcttctggcccaatgctatttcaagatgtctccgcctgcttttgaaaaagggatggaaaaccttacctcttgcgtcacgtcacgctacaagggccgccgcattacggatgccgttattaccaatggctttctggcgatggtggatgccgccattaagaccggcaaatgcagtgagacggtgaagtttgtggaaaactacccttccgtgatgaatatcagtcccacgcgtgtggctttgtacaccccgcggctggtgagctacgttgcggaagtgctggagaaatcccgttccctgcttcaggatggaaagcagaaagagtctgaagattatgcttccctggcgatggtgctgatgggtcttcttcccgatcagtccggagtaatggcggatgccaattattccctggatcgtctgggccgtgccaacggggccgtgcctggcgtgacggatttttcccatacgctggacagagcgaaggtgacggccctgatcgaccagttcaacaagatgaaggaggaaggaaaggtcatggacgccttcacgttcagctttatgggcaaccaggccctggtgcatggttcccaaagggttgcccgcgccgcctaccagcttatcaatgaatcctacccggatgctccgggcagggaggataacctgtattatctggcgatgaccacctggcagctgggagaagcggacaagggaggcgagcttgtggcgcagcacctgaaggaattccccaattccaagtatgcccccatgcttaatacgctgtctttggaagggcttctgaaggaaaaaaaattcgatctctgcgttcagcaggcggacaaggtcatggagttgcataaggatgaccccacccataagttctatgaactggccctgtactgcaaaggagcctccctgttcaacctgggggctgccgacgcctcccgttataaggaagcggtgccggtgctggaacgcttcgtgaaggaataccgtgacagcacttatctgaaaacggccatgtaccttcttggtgaaacctacacgaacctgggcaatacggatgaagccatccggtcctttaccaattacattgcccgtttcccggacaagggggaggccaatatggccgccgtattgtatgaccgggccttcaactacctgaaccgcaagaaccccggagacgaagagcttgccgcgaaagatgcgaaggaaattgtggacaatttcaaggaccaccgcctgttcccgtatgccaacaatttgctggctaatctgtgtgccggcagcaaggagcatgagcaggaagcggaaggctatttcctggccgctctggagtccgccaagaagctgggcgacaagcgtcccgctgcggaagccgtgtacaacctgtttattaacgctaccaagaagcctcttccggtagaaccgaaggaagccgtggaaacggccaggacggcgcgccgggacgaggtcaagaaatggtatgacgagtactggaaagacagcgaccagcccggcagccgctacagcctccagctggctgccgccgccatggacttctttaaggatgacaaggagatgtttgacccggcatccgtcaagatgcaggaaattattgtgagggaaggcaagaaggacgatcccaagatgaccgttcttctggaagaggccgtcaattcctataccaagacgtacatggccggcaatcaggccctgggccgcaatctggatgccaatgccatgcgcaaccacttctaccggttccccggcgtggacaatgataaagacaagacgctgagcgccatgcttcgcatggccgttattgcccagactcaggaacggtatgaaaaggctcctgtggagacggacgaacagcgtgccgagaaagccgccctggaaggtctggtcaagcagctcttcgtggagctgaagcgcgacttcaagccttccgatctgcccccgtacacgcttgtgaagcttggcatgcacctggccggcacttcccagcctgaagaaagcatctcctactttgatgaaatcctggacccgtcggaacctgacccggtgcgtaagaaggcccgcatcaacggcatgtccaagtaccgcaagaatgcggtcttcgggaaagccgtagctctggggcgcagcaaggataacgccaaggtggacaccgccatcaagatgatgagggatgaactgagcaaggaagaatccagctccaacccggaccgcaaggccatggaagacgcccagtacaatctggtcaagttcacttccgcccgccaggactggccggccgtcattgccgctgccgacaagtaccgcgaaaacaagacctataagaagaatctgccggaagtcctctatctgcagggtgaagcctacctgaagcagaatgagctggacaaggcgttgattaacttcatgaacatcacgggtacgtacaaggggctcgtgaagtggtccgcccccgccgtgctggcgcagatggatacgctgtggaagaggaatacgatgtcccagggtgcgggcaagcagccttccgacaggtacgttgcctggaaggccggcagccagtacgtgcagttgctggatactcccgccaaccgcaagaagatgacggcggaggacagtgccctggtcaatgaggtgaaggataagacggccaagttcggttccgatcctgccgtcagccaggaacgggcggacattgccgcctatgaagcagccgtacgcgccgccaagggccagaaataa

SEQ ID NO: 7 - DNA, 1785 bp, Akkermansia muciniphila
ttatttgttaaagttcacgggaatgggcgtttttaacggaagcaccagcttgaagggtacaaaggcccctgccgccgcgtccaccttggcgtccttggctcccagttccatgatctggcgggcttccagtttgacgtctccgggcttgaaagtgaacagggattccttgttcccgtctatttttgcctggaggtcctggatgattctctggccgcccaggctgcgccggacgaatccggtcaggcggatggcgttgacgctgtaaacgcccgcttcatcctcgctggatgcgttggcggaggcctccgtcctgatgtcatccaccagggatgtatttttgtccgatgtgaaggaatccttgatgacggaatatcccgtaatttgggtggtatcctccggattgaagtgggccagcggttcaaaatccgtaaaccagtagggataatccttgtgttccgactgttccagcaggtgcctgatgatgtccgcgtagccgtagcgctgaagcgtgagctgctggtaggaagccagggtggagtccagttttttcagctcctgttctttctggcgcagggcggattgtgccgatttgatggaagtaacggtgggctggacgccggcgaggatttcctccgcctttttctcgcccatatatcctgtgacggcataagctgcggcaccaagaacggcaatggctgccccggcgatgatggcgggcatttttttctggttggcccgctttttggcaactgcggtgggttccaggtcaatattgagggaggccctgccgatggagtgaatggcggtgccgatcaatccgcccaggatgaaggcttcgcgggagatggtgttcacgtccacgccggagcccacgcccacgttgtgcatggggttgaagaaggagatcggaatgcccagtttatcttccaggaattccttggtatagggcagggaagctccgccgccgcacaggtatgccttgacgggagcgcttccgctcatctgggcgcggtaatggttggtggtccgctggatttctgaggcaagcctggtcatggccgtacggatgacggtagccagattggccgtggcgggatccagcccttccgtttgcccgttgctcatggaaacgagcccgctggtggttttcaagcgttccgcttccaggaagggaatattgaattcacgggcgatagcggaggttacgaagattccccccgcggaaatgctgcgggtgaagaaacgtccctgttcgctgtaaatcaaatccgtggatttggcgccgatgtcgatgagcatgaccggttctttctcatccggataactgtccacatacgcattgtacagagaggtaagcgcgcagtccactttgccggtggaaaggccgtgggagacgatttcatcattcagggagtccaggtcttccgccttgatggcaaccaggatggcttcccgttccagacctttggcgggaagcagatggtagtcccacacgacttcgtccagcgggaaggggacgtgctgctgggcttcaaagcggatgagctgttccacatcggtatcgtccagagccggaagcttgacgaagcggatgaaaacggattgtccggaaacggaatagttgacgacgcttcctttgacgttgagttcctggacgaggtcggcgatggcttcccctattttcgtcaggcgcaaaccttctgctgacgggtccagcactacgaggcgcgtagcatagcggtccaggataagggcgtctttggaagtcttggaaaagacgcccat

SEQ ID NO: 8 - DNA, 717 bp, Akkermansia muciniphila
atgaaatccatccttaacactatcacggccatgctggctgcggtgcttttcgtccctgcggcatcggcgcagaccaccagcaatcccagaatgcaggtgcgggtctccctggaaaagctgtccctgtatatgcgccagtcccccaacgtcctgacgcaggacgatccccggccgctgccgaaaccgaagaaatgggcggattttgaaattcccttcaaggtggaagccgctcccacccccaaatccggctatattgatgccctgacgttcaaattctacatcgcggtagtcaatccggaccgctcccgccagtatctgaaactgtataaggaagtcaaatacgtcaatgttccggtaggagaaaacacgtacgcttccgtgtatctctccccgtcctccgtcaagcgcattaccggtgtggaaggaggaagaggaaaatgggtgaagtaccagggcgtagtggtggaatacaacggcaagattgtcgccacttattcctccgaacgcggcaaaatggaaaaatggtggaccatccagtcccccagcatcgtggagacctcttattaccccctgctgaacaaggatgaaactcctttctccgtgttctggtacgaccgttatccggaaattatgaggcccaacagccagcaggcggcttccagttccgtccccgccccgttcggtactcctgtggaacctccggcggacggcgaataa

SEQ ID NO: 9 - DNA, 777 bp, Akkermansia muciniphila
atgtgggtcaaagtatcaatagcagccttggtcattgctcttctcggaggagccatgtattatcttgataacgaggaagctctaaccaaggagcgtagggaatgtgcttcccgctacaagaacctgaacggccttcgtggcgaatttacggaagaaaagacgaaatatgtcgatttcctggtgaagaatgaggctctgacgaatgacatcaatgctttaaccaaggagaaggatgaactggaagtaaagaatcaggaattggcctcagccaatgaggccaagaaatctgaccttcaaacgcagcaaaccgctttggcggaattgcaatccaagagtaaggatatggaaagtatccaagccattgctgacagaatcaaggggctggaagaagagtccaagcagttggaagtggttaagcaggcggaacagggaaaacatgatgccatcgtcgctgaaactgaacagcttgttgtgaataatgccgctcttcgtcagctcaaggccgaccaggatgcccgcctttctccgcccaacctgaaaacgagggtttcccaggtgattcatgattttaatgtagttgtgattgacggaggagccgccgatctgggcgtggtgcccggttccaagttggccgtcatgagggacggcaacaaaattgccgagcttgacgtaaacgctgttgaatcccgtgtttccacggccactattctaccaagtacggtaaccgccggcgaacgtgttgaagccggagacgtcgttgtatctgttcgtccctag

SEQ ID NO: 10 - DNA, 1248 bp, Akkermansia muciniphila
atgagccttcatatagaacccacggaagacgcagtggaaaccctgcgcaaggaaaggcggaaaaattatattgccgcattagcgacatccattctctccgtcgttttggcaggagccattctctactccctgaccatcatcatcgcccctccggaagaacccaaagtcgtcggctacatcacgccggacgatgcgccgccgtcggatacgcctccgccgccggaagtacagagggaaacttcctcttcctcccatgcggagacgcccgtcaaggtcgtggtggcagcggccgccgctccggtgagcctccccaagatcgacattgacccgcccgatgaacctgtcatgctggaggagggaaccgccctcggcatgggggacggcttcggccccgacctgggagacgctacctccgcctttggtacgtccaaaccctccggaagcacgctggtaggtaccttttacgacaccaagcagactcctggcggacgtcctaccaacatgaacatgaaccagtacagggagttcctttcccgcttcgtgaacaaaggctggaacgaatcggaactgaaccgtttttacaaggctccgcaacaattatacgcagcccagttctacatacctaggactcccgccaaagacgctcccaaggcctacggttgcgatgacaaagtaaagcctagccagtggctcgccatttaccggggaaaagtacgcgcccccaagtccggcacgttccgattcgtggggttgggagacgactacttagtagtacggttcaataaacagaatgtcttcgactacggctgggaatccgcttctctggggaaaatgacggcaaacaacgccaaatggcttgatgccatggaaggcaaacccggcaatgacgacttgaaaaaggaactccgggaagtgggcatcaatgtcccccccgttacgttctacaaatacagttcttccgggcactggaacaacactatgcgcggtgtggcagccggcaagcagttcacggtggaacagggcaaggtttaccccattgaaatcctagttagtgaaggtcctggtggcgaattcggcatgactcttctgcttgaagaagttggaatggcccccatgagcaaggatcctaaaacgggagctcccatcctgcccctgttccgaaccaactacggcgttccgaaaccggacaagaacaaggaacacgtgccatttgacgaaatcggcattgtctgggaatccatcaaataa

SEQ ID NO: 11 - DNA, 1383 bp, Akkermansia muciniphila
atgattgaaacgattacagaagaacagttgactccccagcaggccgaattttgggtgcgcgcccgccaggcggtggacatgaacaattatccctatgccgtcagcctgctcaaggccctggtaaagcagctccccggttttctggaaggccgcaaggcgttgcgcgcctgtgaaatcaaattgaatccggaggccaagagaggggggctgttcagcggtatgaaaatcagcaccagcaagctcacttcttccaagaaggacgcggctacccagctttccgctctggaagacgaattggaaaatgatccttacagcattccggtaaacgaggccctgtacacggctgccatggaagtaaatttcccggatctggccgcttttgctctggagaccgttcgccaggggcatcccggcaacaagaaaatgctccacatgctggcctcccattacgtttcccgggatatgccggcccaggctgcggaagtgtaccatgaccttgtgaagctggatcccacggacagtgtggccgtaaagagcgaaaaggactgcatggcgcgcgccacgatgcagcagcagaagtgggaggaggctaaaagcttccgggacgtgatgaagaactcgtcggaaacgaacaccctggacaagagcgacaagaaagggctcacccgtgcggaactggaagagcgcctggggcttctctccgcccgttacgcccagaaccagcaggatctggccgtcgtgcgcgacattgccggcgtttatgaacaaatggaagattgggccaatgcctattccttctataattacgcgttcagcctcagcaacaatgatatttccctggaaaacaaggcctcggaaatgaatgagcgatgccgcaaggcccaggtggaggaaatccgccgccgcgctgccgcggagccggataataaggaacttcaggaacagcttgcccagttcagcaaggaagctgcggagcagcaggtggccttgtgccgccagcgtgtggaaaacaaccccacggacccgcaaacccgttttgagctgggccaggccctcttcgactgcggcaattacacggaagccattccggaactccagcgcgcccgcaacaatccccatatccgcatccgcgccatgctgttgctcggcaagtgctatgacgccaagaacatgcatgatatggctctgcgccagctggaggaagccaataaggaattgatagaaatgaatgacaccaagaaggaaatcctttacatgatcggcttgctttgtgaaaagcagggcaagaagggggaatccctggctgcattccagcagatttacgacgccgagtacggctaccgcgacgtagccaggcgcgtggaatcctcttacggcaattag

SEQ ID NO: 12 - DNA, 462 bp, Akkermansia muciniphila
atgttcaacatcgtgagattcaccaggcgtacctgtccggcattggccctcacgctggcccttacttcgtgcgacagcagtacgaatgaagccctgacctccttcctgacggggaattcatcccaggaacaccagcagctccaggcccagctccagcaaatgaaaaacgcactggcccagacggaacaggaaataagccaggcggaatcccacgatgcccgcgttaattacaatcttcagaaaaggctttccaacccgggaagaatcacgacgcccttcacggtgaaggatatagatgtcctgccttccaaacgccgcgacttcgagcacctgtgctttgacattgaagacatgcgcaaaacgctggcgcagcgcaagcaggaattccatgccctgcaatatcaatataacgcgtatgcggccaaactggctgaattcaaacaaacccacccggtagactaa

SEQ ID NO: 13 - DNA, 747 bp, Akkermansia muciniphila
atgccaaaaatcgttgttcaatcctgcatcatctgtatgagatatttttccaagcattccggaatggctccgcgctgttcctcgccggggagcaaggggtttaccctggtggaattgattgtcgttatcaccattatggttgccatgatggccttggccgccagcatgttgaggggcgggggcagggggcaggggcttcaggccgccgttgaaatggtggacggcatggtgcaggaggcgcggctggatgccatgggcaaaggaacgtggagccgcctgattattgtgagcactcccgatgacgaagcccgcaatatgcgcactttgggcgtgatgtccaaaaatacccgcaccgggaaatggcatctggtgaaccgtttgcagactctccccgccggtttttacgtcagtccggcctacagcacccttctggaaggctcgaagaaagccagaggcgagaaatccacggcccgcggttttgccagccgtgacgggcaggataccgtcaaccttcccggcaacagaatgacggatatttacttcattgaatttgacgaggaaggccgcatgtcccagccgaacgcccccacccgcctggtggtggttgccggttccgccggaaacggcaaggaggagaggccgaccccgatggtggacggcaaaccgggcctggcaggcggcattgtgatttatcccaaaggcaatatcagccgtctgaggacgacggagcaggtgattcccaattag

SEQ ID NO: 14 - DNA, 801 bp, Akkermansia muciniphila
atgttgaccaagtgtatgaaacagtctcgtgccaaggggttcaccctgacggaagtggtgcttgcgatcggcgtggtggccgtgctgattgtagtgttcatggccatgtttattcctgccagaaggacggttcagtccgccctgactattcgtgaagcggaccgcatcgtccacgccctgacggcggaacttggagaactccgcaattccgagcgtgccgcgtccaacgccagaaagtcttcctcctccagatatgtttccgcttttgacaaggcgttttactggatgcagttcacgtccaggcccgctacgaccattcttgtttacaattacagggcggatttgaccaagggggcccgcaaagacggaactccccagccctggctggaggatggcggaagcattcccggcaaaaatactgcggtggtgacaggggtctgcctggcgaacaacaaagagcgttgggatgatttcaaggcccttgtcggtcccgtcttcgccgtgcgcatgacccagctggtagtggagcgcatggattcaagctcctacgggtacaagctggctcccaagtacgggacgatttataatccttacaaccgcggcaaggtgattaaggaaccttccctgtatgtttatacgccggagaaaggcggcggcctgaatttgccgtggggggcggaagtcctgtaccaggcggagttcttccagctgttgaatacggaccccgagcgtttacaacatctgacgtgggaaaatttaaagactcccgtgtttacgcgcaatctcgctttccgccgttag

SEQ ID NO: 15 - DNA, 759 bp, Akkermansia muciniphila; identical to SEQ ID NO: 4

SEQ ID NO: 16 - DNA, 3234 bp, Akkermansia muciniphila; identical to SEQ ID NO: 6

SEQ ID NO: 17 - DNA, 1659 bp, Akkermansia muciniphila
atggacaccaacctcacactggaacttttcatcggccggggaatgattgacaaatccctggcaaaggacatcaaggaggaaatgatcgcctccggcaaggagctgccggaagtgcttgcagacttcggcatcatcggcagcaaggatgatatctggcagatgattgccagcgacctgggtacggaattcattacactggacaacttccagccggatccgaacgtgcagaacatgatgccggccacgctcgtgcgcctgcacggggcgctccctgtgcggcatggtccggaaggcctgtacgtctgcctggtggatcccctgaatccccagacggtggaagacctgcgcttcgccctcggccaggacatccatgttctggtagcgccggattaccagatttccgaacgcatcaatgagctttatggaggcgaatccgccgccatgtccgacctgatgcaggagctgaacaacatgcaggtcaacaatgagacggaggactccgccgccgctcccgtcatccgctttgtggacctcgtcattacgcaggccatcaaggaaaaggcctccgacattcacttcgaaccttttgagaaggaattcaaaatccgctaccgtgtggacggcgccctgtatgaaatgcagcctccccccgtccacctgtccgtgccggtcatttcccgcgtcaaagtcatggcgaacatgaacatcgcggaacgccgcattccgcaggacggacgcatcgtcaagcagataggaaaccgttccgtggacatgcgcgtttcctcccttcccactcagtacggagaatccgtggtgctccgcgttctggaccgctcttccgtcaacttgaacatggacaacctggggcttcccgcgcatatccacgaatatattctggatacggtccacaagcccaacggcattttcatcgttaccggccccaccggcgccggcaagacaactacgctgtatgccgccctgcgtgaaatcaataccattgattccaaggtgctgacggcggaagaccctgttgaatacgatattgacggcatcatccagattcctatcaatgaagccatcggcctggacttcccaatggtgctccgcgccttcctgcgacaggacccggaccgtattctggtgggggaaatgcgagacatggcaacagcgcagatcgccatccaggcatccctgacgggtcacctggttctctccaccctgcacacgaacgactccgccggagccattacgcgactggtggacatgggatgcgaacctttcctggtggcggcttccctggaaggggtgcttgcacagcgcctggtgcgcaccatctgtccggactgccgcacgccgtatgaaccctcatccaccatcctctcccagcttggcgtctctccctatgaactgggagacaagcactttttcacgggccgaggctgtgataaatgctccaattccggctacaggggccgcaaggggatttatgagctcctggatattaacgataccctgcgcgacatgattacggatcgcgctccttccgtggtgctgaagcagaaagccattgaaatgggcatgtccacgctgcgggaagacgggctgagaaatatttatgacggcaacaccaccattgaagaagtgctgaaatatacttaa

SEQ ID NO: 18 - DNA, 1269 bp, Akkermansia muciniphila
atgcctaaatatcaatacacagcacttgaccataaaggcgaccagaaaacaggtaccctggaggccaattccgaagcggaggccatggaatccatccgggcgcatggcctgtaccccacccagatcgtagaagcgggcaagggcaagattcagcagacgcctgccgccaagaaaaaggccaagggagccaagaagcaaaaaggcaagctgggaggcaaaatcaaggccaaggctctgatgattttcacccgccagcttgctacgctgattgacgcggggcttcccctgctccagagtttgaacgtgctggccaaacaggaggcaaaccccaacctgcgcgtaaccattgaggctcttggagattccgttcagggcggctccaccttctcggaagccctggcccaacaccccagaatttttgaccgcctgtttgtcaacatggtaaaggccggggaactgggcggtgtgctggaagtcgtgctgaaccgtctggcggaataccaggaaaaggcccaaaagctgaaaagcaaggtgatctccgccatggtgtatccctccatcgtcctgtttatcgccgtaggcatcgtgatcttcctgatgctggtcatcgtgcccaaattcaaggcgatgttcgcagaacagaaccaggaacttcccggtatttccgagtttgtgttcggcatcagcgactggttcatggccgcccccttctttgtgcccaatgccgtcattctggccgcggtagtcgccatcctgtacgctgttttcacggccatgagcaagacgcccaacggacgccgcaagattgactccgctctgctgaccatgccggtcatcggcaatgtgcagagcaaaagcgccatcgcccgcttcgcccgaaccttcggtacgctggtgacttccggcgtccccatcctccaggcgcttaccatcacgaaggataccgccggcaacatgatcgtgggagacgccatcggcctcatccatgactccgtcaaggaaggcgaatccgtagttacgcccatgtcctcctccaagcttttcccgcccatggtaatctccatggtggacgtgggggaagaaaccggccagttgccggacatgctcctgaaaatcgcggacgtgtatgatgatgaagtggacaatgccgtgggagctatgacctccatgctggaacccatcatgatcgtattcctggccgtggtcgtgggcggcatcgtgttcgccatgttccttcccctcctgcaggttattgaaaagatgggataa

SEQ ID NO: 19 - DNA, 717 bp, Akkermansia muciniphila; identical to SEQ ID NO: 8

SEQ ID NO: 20 - DNA, 984 bp, Akkermansia muciniphila
atggacacccgagaattcaacgaaattatcgccgcgaactcatcgtggatttctgctctcagaacggaagtcggcaaggtggtcatcggccagcaggcgctcgtggacagattaatcctcagtctcctctgcaagggccacgtcctgctggaaggcgtgcccggccttgccaagacgctctccgtaaaagccatggcgggcacgctgcatgcacagtttgcccgcatccagtttacgccggatcttcttccggcggatttgctgggcacaatgatctataatccggaagaaaggcagttcacagccaaaaaaggcccgatcttcgccaatctcattttggcggatgaaatcaaccgcgccccggccaaagtgcaatccgccctgctggaagccatgcaggaacgccaggtaaccctaggtgaaaccacctaccgcctgccggaccccttcctggtgcttgccacgcagaacccgattgaccaggagggcacttaccagctcccggaagcccagcttgaccgttttctcttcaaggtgctggtcacctaccccacgcgcgaagaagaactccaggtgctggacctcatggccagctccgccaaaccgccggaaacctccccggtcaccacgccggaacaggtggcggcctcccgcgacctggtaaaccagatttatattgacgacgccgtgcgcggctacatcgtggatctggtgcgcgccacccgcttcccggaaacggtggacgtgaagttgcgcggtctcatccgcgcgggggcatctccccgcgctaccatcaacctggctctggcggcccgcgccaatgccttcatgcaccatcgttccttcgtcactccacaggatatcaaggacctggcccacgatatcctgcgccaccgcatcctgctctcttatgaggctgaagcggaaaacatttccacggacgacgtcatcgaccacatcctgacgaaagtccccgtgccgtga

SEQ ID NO: 21 - DNA, 462 bp, Akkermansia muciniphila; identical to SEQ ID NO: 12

SEQ ID NO: 22 - DNA, 1383 bp, Akkermansia muciniphila; identical to SEQ ID NO: 11

SEQ ID NO: 23 - DNA, 468 bp, Akkermansia muciniphila
atggaaaatacatatcgtcatgcccagcttccggaagggcgcgttcccgccctgcgcgtggaaccaatgcctgcggataccaatcagagcggggaagtattcggcggctgggtgatgagccaggtggaccttgcaggagccaataccgccatgcgctatgcattgagccgctatattgtgacgcgtgcggtgagcagcctgacgtttgaagctcctgtgctggtgggcgatgtagtgtccttttatacggatattatcaaggtgggccgcacctccgtcaccgtgaaggtggaggtgtatgcggaacgtctgacgaagctttgcaataacattgccaaaattacagaggcggagctggtttatgtagccctgggggaggataagaaaccgattaccctggaagagtcccgcgcccggtttgcgcagtgctgttctcttgagacgggagattcctcttcctgttcctga

SEQ ID NO: 24 - DNA, 1413 bp, Akkermansia muciniphila
atggggaaaacgcttttccaaaaaatctgggacgctcataccgtcggcatcctgccggatgggagaacgcaaatgttcatcgctacgcacctgctgcatgaagtcacctctccgcaggctttcggaatggtccgggacctgggcctgactgtgcgccacccggaacgcacctttgccactgtggaccacatcattcccacagacaaccaggcggaaccgttcgcggacgccacggctgacgccatgatcagggaactgcgccggaactgcgctgaaaacggcatccgctttttcgacctccctaccgggctccagggcatcgtgcatatggtagggccggaactcggcatcactcagccgggcatgactatcgtatgcggagactcccatacggccacccacggagccttcggtgccattgccatgggcatcggcaccacgcaggtgcgcgatgtgctggctacgcagaccctggccctcagcccgctcaaggtgcgccgcatcaatgtgaacggaaagctggcccccggcgtgcgcgccaaggatgtagccctgcacatcatcggccttctgggagccaagggcggcctgggcttcgcctacgaatacggaggcgaggtcattgacgccatgagcatggacgaacgcatgaccctctgcaacatgtccattgaaggcgcggcgcgctgcggttacgtgaaccctgaccggaccacggtggaatacatcaaaggacgcctgttcgcccccaccggcgcggactgggacaaggccgtggaacgctggctgggctttgcttccgacgcagatgcggaatatgatgaaatcgtggaaattgacggagcttccattgagcctacattgacatggggcatttctccggaccagaatacgggcatcagcggcagcactcccaacccatccgacgcagcggacgacgatgaacggaagatgatcaatgaagcgctggaatacatgaaattccccgcggacatgcctcttaaggggctgccggttcaagtgtgcttcgtaggttcctgcaccaatgggcgcatttcagacttccgggaagtggccgccctcatcaagggtcgccatgtggcccccggcatcagggcgctggccgttcccggctcccagatgactgcccggcagtgtgaagaggaaggcatcgcggacattttccgtgaagccggctttgaatggcgtctggcgggttgctccatgtgcctggccatgaatccggacaagctccagggtgaccagctctgcgccagttcctccaaccggaacttcaagggccggcagggaagccccaccggacgcaccctgctgatgagcccggccatggtggccgccgctgctctgaccgggaaagtctccgatgcccgcgaagtgttctccctgaattaa

SEQ ID NO: 25 - DNA, 1785 bp, Akkermansia muciniphila; identical to SEQ ID NO: 7

SEQ ID NO: 26 - DNA, 2961 bp, Akkermansia muciniphila
atgttcaccaatattacacgcacgaccctctgcattactgcgttcagcatcgccagcctcatggcggcgcctctgaatgcaaccaaaacggagagcctggattggaactggaaattcgcccgtttcgggaaaatgccggatggcagtacgcaaccggaaccgggaaaagccatgggattcgccactgccaccagtgaagaatccggcaatccggcggacaatgccgtggacggggacaagtccacccgctggtgtgccgccagtggcaaaagcggagaaaaaatcaccgtggacatgggacgccccgtagatgtaaaaaccgttaacatcctgtgggaaaaacaaagcaaccatcttttcaagctggaaggctccggtgacggaaaacgctgggcaactattgaagacaaaacttccgggcaaaacgactccaaggaagacacggtagaaaacaaaaccggcaaaccgcgatacttccgcatcaccgtcacgggcaacaaccagagcaactgggccagcatccgtgaaatcacctttaaaaacgacaagggggaaattatccgccctcaggccgccgccggaaccagtaaggcggacaatccctccagcccctctttcaacgacaaaaactggcgttccttgaacctgccgcacgactggggcgtggaaggacccttccggatggaaattgaaaacagaaccggaaaactcccctgggtcggcattggctggtaccgcaaaacgctggaaatcccggcggacgccaagggcaaccaattctatctggactttgacggcgttatgtcccgccccaaaatttatgtgaacggacacctggccggcgaatggaaatacggttacagctccttccgcgtggacatcacgcccttcctgaaattcgggcagcaaaataccattgccgtcagagtggacaatccccccagcacctcccgatggtatccgggcggcggcatctaccgccatgtgtggctcacggaatccaaccctgtgcacatcgaacactggggcgttttcgtcaaaactccggaaatcaccaaatccgccgccaaggtagaagtggacaccacggtgaaaaacaccacggacaaagccgtcatccccactgttactgaagaaatcctggacggaggtaaaatcgtagcctccacaaccaccaaaggggaagaaattcccgccggggaaaagggcaaaatcaccagtacgctgacgctcaaaaaccccactctgtggacgctaaacgctccccatctgtataagatgaaaaccacggtcaggatgggagacaaagtcatagaccaaaaattcaccaacttcggcgtaagaaccgttgaatggaaacccacgggattctaccttaacggggagcgcgtgcagctcaagggcgtttgccagcaccatgacctgggaccgctcggctccgccgcccacacgcgaggctatgaacgccagattgaaatcctgaaggaattcggcgtcaactccatccgcacgtcccacaacccgcctgcgccggaagtgctggacctgtgcgataaaatgggcatcctggtcattgacgaacttttcgacgtatggcaatgctccaaagaaggcgtcaacaacgaatcctttaacgaatggcatgaacgggacgtggttaacctctgccaccgggaccgaaaccacccctgtgtcattgcatggagttcgggaaatgaagttccggaacagggaatgaaaaatctgcaccatatctcccaaaccctgacggatcttttccaccgggaagaccccacgcgtaaagtgacttccggctgcaacaacgccaatgccgcacgcaacggctttggggacaccctggatgtttacggctataactacaagccctgggcctacaaggacttcgccaaggaccgcccccaccagccgttctatggtgcggaaaccgcctcctgtgtcagctcccgcggagaatacttcttccccgtggactggaacaaaggcaagggattctacctctaccaggtcagttcctatgacctgtacgcccccggctgggccaaccgtccggatgtggaattcgccgctcaggaagacaatcccaacagcgcgggagaatatgtatggacgggctttgactacattggggaacccaccccgtacaatctggacgccaccaacgccctgaacgtgccggaagggccggaacgcgaaaagctgatggcggaactcaaaaaactgggagaccgcgccccctcccgcagctcctacttcggcatcgtggacctgtgcggcttcaaaaaggaccgcttctacatctaccaggcccactggaggccggatctcaagatggcgcacatcctgccgcactggaactggccggaacgcaaggggcaggtaacgcccgtgcatgtctacaccagcggggatgaagcggaactcttcctgaatgggaaatcccagggcgtccgcaaaaagggcaccggggaaaaggaccgctaccgcctcgtgtgggaagacgttaaatacacgcccggcaccctcaaagtagtcgccaaaaaggacggtaaaatctgggctacggacacggtaaccactaccggaaaacctgcggcgctcaccctcaagccggaccgcaatgaaatcaagggagacggctatgacctgtcttatgtcaccgtagccgtccgcgacgcccagggccgtatggtgccccgaagcaaaaaccagctcaccttcaaggtaagcggccccgcggacatcgccggcatctgcaacggtgatcccacggacttcaccaccatggcgaatccggaaaacaagaaaatcatgaaaatcaaggccttcaatggtcttgcccaggtcattctgcgctcccgcaagggagaatccggaaaagtgacgctccaagtcatctccaacggactcaagccggctcagacaactgtgacggtcaaataa

SEQ ID NO: 27 - DNA, 1161 bp, Akkermansia muciniphila
atgaatgagaaatcgttgattccgtctatccgctttgccggatttactgacgcatgggaacggcgtaagctgggggatttagcggagtttagaagagggctaacctattcaccaagagatatatcaacatctggaatcagggtattgcgctcgtcaaatatagatgaggattctttcgttttagcagaggatgatgtttatgtaaaagagacggctgtgtgcatcccgcttgttgaaaaaggcgacattttaattaccgcagctaatggctcaagcagattagtcggaaagcatgctttgattattgacgataagggtaaaatggtacacggcgggttcatgctgctcgcgcatccgtatacgcattctgctttcgttaatgctcttatgcatgcaccctggtactcatcgtttatccgcactaacgttgctggaggaaatggagctataggaaatctgaataaaagcgatttggaagaacaagatattgcggcgacctctgagcaagagcaagaaagaatcggttccttgtttgcctccctcgaccatctcatcacccttcatcagcgtaagtatgaaaagctccttaacatcaaaaaatcgatgttggacaaaatgttcccgaaaaatggtgagcttttccccgaagttcgctttgccggatttactgacgcatgggaacggcagaagctgggggatttggtagagtctgttccgtttaagcagtatatagcatcacctgaacctgacggaaaattcgaaattatccaacaaggaagtgagcctattattggatatggaaacggaatcccttgtgaagattatgcaaagataacgattttcggagaccatacagtttcaatctacaaaccacaaaagcccttttttgtagccactgatggcacaagactccttacagcaagagttctagatggagattttttttatttcctcttggagcgatacaaaccaatccctgaaggatataagcggcattacacgatattgattgaaaggtatggatgttttccttcccatcgagagcaaaagttaattgccatattttttaggaacatcgaccacctcatcacccttcatcagcgtaagttggaaaaactgcaaaacatcaagaaagcctgtctggaaaaaatgtttgtttaa

SEQ ID NO: 28 - DNA, 564 bp, Akkermansia muciniphila
gtgaaaggatttttttgcccgttttcaacgggtttatggaaggaacatggctggaaatgcggaaaagggtatgttaatgaacagggcatggaaagattgtatcgtccgaatgttgcggggatgatggtccggcaggacgggaaattgttgatttgcgagcgttccgggcagaaaggagcctggcagtttccccagggcggaattgacccgggggaaacggctttggaagccgtgcggcgcgagattggggaggaagtggggtttttgccgtcccagtataatattgtggaatcccggaaggggtatcgttacgattatccgccggaggtgctggagtatgttcgtgaaaagcggcggcagccttttgttgggcaggcgcaggagtatttcctgtgctggctgcatgcggacgctccggaacccgtcctggatgaccgggagttttgcgattacaagtggatagccccagccgaatttaagctggagtggctgccggagtttaaaaagaaagtttacgccagggttctggaagatttctttaatgtccgggcgcgggataagtaa

SEQ ID NO: 29 - DNA, 1422 bp, Akkermansia muciniphila
atgtctattttctcatcacgcagacaatttctcaaatctttggggcttgcggccggagcggctgccgccggaaatgccctccctgggaaggctgtggaaatccctgccggagaccatctctggaaatccgcctctccggcggctccgaggccttccggttccacatacatgggagggttcaaggctccccggctgggtcgcatcaggctggccttcatcggcgtgggagggcgcgggttctcccacctggcgcaaatgtgcgtgatggatggagtggaaatcgtgggcatatgtgatttgaaggaagagttgacgaaacgcggcgtggatcgcgtgctctccagaatggggaaaagccctttgggctattccggcggcgatatggaatacctgaccatgctgaaggagctgaagccggatgccgtcatcatcagtacggattggagttcgcatgccagaatcgcctgcgacagcatgaagcacggcgctcacgcctttgtggaagttcctctggccgtctctctggaggagctctggagcctggtggataccagcgaggccaccaggaaacattgcatgatgatggaaaacgtcaactatgggcgggatgaactcatgttcctgaacatggtccggcagggcgtcatcggcgatttgcttcacggggaggccgcgtatatccattgcctggtgacgcagctgggggacacgcgcggggaaggggcctggcggccggaatatcataccagaatcaatggcaacctgtaccccacccacgggttggggccggtggctcaatatatgaatttggagcgtggagaggaccgtttctgccgtgtggcggcgttcgcttctcctgctctcgggcgcaatgcctacgctaaaaagcatcttcccgccgatcaccgctggaacaatactccattcatctgcggtgacatgaatacggctgttgtcaagacgcagctggggcggaccattcttgtccagctggatgagacgtccccccggccttactcccgcgccaacctgatccagggaacggagggcacgctggctggtttcccaacccgcgtggcgggtgaaaagctgggcaacggcaattatcatgaatggattgaaggcagggaaaaactggccgctatttatgaaaaatacgatcatcccctctggaaacgcatcggggagctggccacgaaaatgggcggtcacggcggtatggactttgtgatgctttcccgcatcgtggaatgcctccggaacggagaaccaatggatcagaacgtttacgaaggagcttcctggtcttccctgctgccgttgacagcccgttccatcgcccagggcgggatgcctgtggaatttccggattttacccgcggagactggaaaaccaccatgccgctggccgtggtttcatga

SEQ ID NO: 30 - DNA, 816 bp, Akkermansia muciniphila
atgaaaactgtcttagtagttttattgattcttgcagcaggggcgggcgcctggttctccggtcttagcggccttttcggtattaatggccagtatcaggattttaaagaaatgatttcgtatcgtaagactttggacaaggaaatacgtacttggacaagcttgcgcaacgacatgattaagaatcgtggcttggcagcggaagaaaatcttagtctgatttccaacaaggcttccgtgacgcagcagcgtgatgaacagctttccaaggaagcggagttgaaggaagaagaagtgcagttgaatgcggacttgtccaaaatcaataaacagattgaggaattaaagagcaagttgcaagatttcggtgtttccagcgtacaggaaatccaggagaagatggaatctttggaagcttccaataagaagctccaggaagatattgaccagattaaaagtgctacggaagtggcttccaagagacgggcagaacaagcttctgagctggctagccgccagaaggagcaagctgaataccgagctgctcttgccaaaaatggggaagagtatcccgttctatccgtggatccgcagtggggttttgttgtgattggggccggacagggcagtagtattgatccaaatacggttcttcttgttacccgtgaaggtcgcagcattggtaaattaaaggtaacttccctggagaaaaatcagacggtagctgacattattaaagacagcgtaccgtctggtatgagtattcaacccggcgatagagtacaactcctgcgtccccgtcagtccgccaaataa

SEQ ID NO: 31 - DNA, 429 bp, Akkermansia muciniphila
atgctggacttgagcgcttctctttccacggaagatgggctagggccgtggaatattatcgtcaaattgacgggcaatggttcggaccttccccaggtaagcattaatgcggcaagcagcaatgaaagtgctcctatgaacattgcttccgtagtgtaccgcaggacgggatcatccgctattctgagggggaacttcacgattacttccgggcagtggacggctccgggcccgattgtcgtgacaaacagggacaaggcctttatagatgctaatatttccttcagttcctccaatgaacgtgagagctgcggcgggacgttcaccggttccatcacttaccaggttcccgttgagaatgatgaaggcgaggttgaagcgcaggactggaccgctacggaaggaacggtgagttacacggtatcctga

SEQ ID NO: 32 - DNA, 1446 bp, Akkermansia muciniphila
atggatagcattctttccgtccttgccactatcgccattattttcggcgtggtgatgttgtttaacttcatgatttttattcatgaacttggtcattttttcgctgcccgctggcgtggtctgtatgtggacagatttcaaatctggtttggccgtcccatctggaaaaaaacggttaacggcgtgcagtgggggctggggtggattccggccggaggttttgtatccctgccgcagatggctcctatggaggccattgaaggacgtgcggagcttcccaaggatttgaagccggttactcccttggacaagattatcgtggccgccgctgggcctgccgcttcttttctgctggctgtgttgtttgccgtggccgtctggatggtgggcaagccggatgtggagatgggcgtgactacggtcggttttgttgctccggacagccctgcggctcaggccggcattcttcccggcgacaagattgtgaaagtggacggccatcctgtggacaagtgggcgggcaatatggaaggcgtgcgggaattgatcatgctgggcgagcatgaccgggtggtttttacggtgcagagacctggacatgaaggagagatggaaatttcctgcggattccggattccggaaacgtcctggtggcagcgctccggcatgcgtcaggtggggttgatgcaggccatgccctgcgtgattggggaagtgattcccaattctcctgccgcactggccggattgaacccgggcgataaggttgtgggtgccaatggagaacgcctctggaaccctgccgcactggatgttctgctgaagaagaatgaaccgctcttgctggatgtgacggacagggccggggttgcaaggcaggtgaatatccaggggaagcttccggagaattggcacaatggtgcggacggttccctgctcaagggggcccagcctattctgggcgtgagctgggacctgagttccgtgggccgagacgttaccgtccatccttctccgtgggcgcagatcaagcagagtctgaaatggatgggggataccctggcgaaggtggtggctcccggcagcagcgtgggcgtggagcatctttccggacctgtgggaattgccaatcagttttacaagatgttctctctggaggaagggtggaagctggccctgtggttttccgtggtgttgaacgtgaacctggcggttctgaatattctgcctcttccggtagtggatggcggccatgtggtcatgaatgccattgaattggttttccggcgtcccctgaatgtaaaagttctggaattcgtccagttcggctttgtgttcctgctgatggggttcttcctgtttgtgacattcaaggatgtgggggatttctttggcaagaagccggacaagctgcccaccccggtattcaaggccgtcgcggattag

SEQ ID NO: 33 - DNA, 927 bp, Akkermansia muciniphila; identical to SEQ ID NO: 2

SEQ ID NO: 34 - DNA, 1200 bp, Akkermansia muciniphila
atgtatacccccgaattcaaaaacatcctcacttccaccctggacggactgcgtgcggaaggactttacaaggaagaacgctttatcgcctcccagcagtactcccaggtgacgctgaaggacggacgctccgtcatcaacatgtgcgccaataattatctgggccttgctaataatccggaagtgatggaagccgccaagaaagccatcgaccagtggggtttcggcatggcgtccgtgcgttttatctgcggcacgcagacccttcaccgtcaattggaagaacgtcttacccaatttctcggcacggaagacacgattctgtttccctcctgctttgacgccaacggcgggctgtttgaaggcctcctgactgcagacgacgctattatttccgattccctgaaccacgcttccattattgacggcgtgcgcctctgcaaagccaagcgcttccgttatgccaacaacgacatggcagacctggaagccaagctccaggaagcggacgccgccggagcgcgcgtgaagttgatttccacggacggcgtcttttccatggacggcatcattgctcagctggacaagattcacgagctggcagccaagtacaatgccattgtccactttgacgactgccacgccacgggcttcctgggcgaaaagggccgcggcacgcatgaataccgcggcctgttcggccatatagacatcaccaccggcaccctgggcaaggcactgggaggcgcttccggcggctacgtctccggcccgaaagaagtagtggatgtcctgcgccagaaggcgcgcccgtacctgttctccaacagcgtggccccggctatcgtagccgcttccatcaaagtactggacctgttggaacagtccacggaagcgcgcgaccgcgtagaagccaataccaagtatttccgtgacgcgatgacgggagccggattcaccatcggcggcaaggaccaccccatttccccggtcatgctgggggatgccgtcctgtcccagaaattctccgcccagcttctggacgaaggagtgtacgccgtcggcttcttctatcccgtcgttcccaagggacaggcccgcatccgcacgcagatttccgcagcccatacccgcgaacagctggacaaggcgattgaggccttctgcaaggtaggtaaaaacctgggcgttatttcctga

SEQ ID NO: 35 - DNA, 2745 bp, Akkermansia muciniphila
atgtccaccaattcctgcgcgtgtagcgcatctactgacaaattcgtctattctttcggcggagggtccgccgacggcaatggcagcatgaaaaatcttttgggcggcaagggcgccaaccttgcggaaatggcccgtatcggccttcctgtccctcccggattcaccatcactacggaagtttgcacttactactacgatcacggctgcacttatcccgcccagcttgacgcgcaggtcaaggaaggcattgccaaaatggaacagatcctgggacgcaagttcggcgatacggaagctatgcccctgctggtggccgtgcgttccggcgcccgtgaatccatgcccggcatgatggacacgattttgaacctcggcctgaatgaaaaatccgtggaagccatggtgaaggctacgaacaacccccgcttcgcctgggactgctaccgccgcttcgtgcagatgtacggcgacgtggtgctgggtgtgcagaaaaccccggatgaagaccacgaaccctttgaaaccgccatcgctgccatcaagaaagaacgctttggcagcgaggacgtggaagacaccaagctctctgccgatgacctgaaggaacttgtctcccgcttcaaggccctggtgctggaacgcaccggccatgaattcccggaatgcccctgggaacagcttcagggagccattggcgccgtgttcggttcctggaacaatgaccgcgccatcgtgtaccgccagaaatacggcattccgtccgaatggggcaccgccgtcaacgtgcaggccatggtcttcggcaacacgggtgaggaatccggttccggcgtggcgttcacccgcaaccccgcctccggcgaaaacgaattctatggcgaattcctgatgaacgcccagggtgaagacgtcgtggccggcgtgcgtacgcccgcccccgttgctgcccttcatgaagtgatgcccgccgccttcaatgaactggtgcgcattcgcgaagtgctggaaaaccacttccatgacatgcaggactttgaattcaccattcaggaccgcaccgtctacatgctccagacccgcaacggaaagcgcaccggcgtggccgctttccgcattgcctgtgaaatggtggaacagggcctgattgactggaaaaccgccgtgcgccgcattcctgcggaccaggtggaccagctgctgacccccatctttgaccgtgaagccatcaagagtgccaaggttctgacccgcggtcttcccgccgggcccggcgccgccaccggacgcatctacctgaacgcggaacgctgtgtggaagccgcggatagaggtgaaaaggttctgctggtccgtctggaaacctctccggaagacctgcgcggcatgattgccgctgaaggcatcctgaccgcccgcggcggcgtttcctcccatgccgccctcgttgcccgccagatgggcaaagtctgcgtttgcggcgcggatgaaatcattgtggactacaacaaccgcaccgtttccgttggcgacgtaaccatcagcgaaggtgactacctctccattgacggaacgagcggcctggtatacgccggcaaggtggaaacttccccctctgaaatcatccaggtcctgatttccaagaccatgaagccggaagacagccgcacctaccagaacttcgccaagctcatgcagtggtgcgacgactgtaccaaaatgaaagtgcgcaccaatgcggactctcccaagcagacggaaaccgccatcgccttcggcgccaccggcatcggcctctgccgcacggaacacatgttctttgaaggggaccggatcgacttcgtccgtgaaatgatcctctccaccaagaagagcgaccgcgtagccgccgtttccaagctccttccctaccagaagggggacttcaagggcatcttcaaggcgctcaagggcctgccgggcaccatccgccttctggacccgcccctgcacgaattccttccccagacgaaggaacagcagcttgacctggcccagaaaatcggcatgcctgtggaagttatcatgcgccgcgtgtccgaactccatgagttcaacccgatgctcggccaccgcggctgccgtctcggcatcgcctatccggaaatcacggaaatgcaggcccgcgccatctttgaagccgctgtggaagtctcccaggaagaaggatttgccgtggtgcctgaaatcatggttcctctggtggccttcaagaaggaactggacatccagaaagccatcattgacaaggtggcccagcaggtatttgaggaaaaaggcgtcaaagtggactacctcgtcggcaccatgattgaaatcccgcgcgctgccgtcacggctgacgaaatcgcggaaaccgcccagttcttctccttcggcaccaatgacctgacccagacgggcctgggcatgagccgcgacgactccggctccttcctgccgcagtaccaggaactggaaatcatcaagaagaacgtcttcgcttccattgaccagaacggcgtcggcaagctgatgaagattgccgtggaactcggccgctccacccgcccggacatcaaactgggcatctgcggcgaacacggcggcgaccccgcttccgtcaagttctgcaacacgctgggcctgacttatgtgagctgctcgccctaccgcgtcccgaccgcccgtctggccgcggcccaggctgctctggaacaggaataa

SEQ ID NO: 36 - DNA, 885 bp, Akkermansia muciniphila
atgcgtcttttatcctccgccgccgtcatttgcgccgccctgttctccggaaccatccttcatgcgcaggacccggaactgctggccaagcgccagtgccgttccgtccatatcaaccagcaggggcatccctcccaggcaagcgccctgtacaatgtagtgaaagccaaaacatccgttcccggcacctacttttgcgccatgaattttgacgacggctatatcggttttcaggaacaatccaacggtaaaaaagtaatcatcttttccatctgggatccggtggcacacggagacaaccccaatgatgtgccggaagaagaacgcaccaagctggtaaaactgggcaaagatgcgcgctccggacgttttggcggtgaaggaacaggcggacaaagcttcgtggactatccctgggcaatcggggagaacatgcgcttcctcgtctgcgtcaaaaaaatggggaaattcaaggaaatcagcggttattactttaataataaaagcaggtcctgggatcttatttccaaatggaaaacgcattcctcggaaaaggaactttccttctccgtcggattcgtggaagatttcatgcgtaattttgaatcagccaagaaggcccgcggagccttctttggccccagcttcgcgtacaaggacggcaaatggcatcccaataccagcgtaacgttcaccggcgacccaaccccctccaccaacgtcatggcgaacatccagcctgatggttccgtgctgcttcagacggggggaactacgaaaatgacggatttcaagctgttccaaaatcgtcccctgccccagaatatcaagctggtcctgcctgacaaggccgttaccagtcttgttcaggagaacattaactga

SEQ ID NO: 37 - DNA, 870 bp, Akkermansia muciniphila
atgatagataagacgacatcccgcgtcattatggggcttttgggaacagcctgtgtcttgattacggcatttgcctggtacaagacgaaatatgccgccgttccggaggccgggatgcaccataatatttatgacgaagacattccgcggtctgctccggttcctgtagattaccggatggttttgttgacgccccaggagctggcaaaggcgcctctggccgatgtgtttacatcgcccctcggagatgagaatggagcgtttacctatgttgcccagggtgtgggggatatgaatgccgcccgtaagggaaggcatgcaggacaggatttaaatggaataggaggagaaaacacggatgagggactgcccgtgcgggccgccggccgcggattgctgatttatgcaggagaaccttctccagattggggcaatgttgtcgtgctgctgcaccgcttgccggacgggcgttttgtgcagagtctgtatgcccatttgaaaaccgtcagcgatattccgctggggactctggtgggacgcggagagcaaatcggctcagtcggaactgcgcacggcaattatttggcgcatttgcattttgagatgattgaatccatcgctcatgaggcgggaatgccgggctatgggaagacaacgtttaacagaatcaatccggatgaggtgctaaagcaatatgctcccgacccggaaatgatgatgcctgatcctattattgccttgaaacaggttcagatggcggcggggtgggaaaaactgctggagaatctgtataaggataacagcatggaagctttggataaaatcctcccagacagtcagccgcccacggaagaaaaggaaaaacgctga

SEQ ID NO: 38 - DNA, 2619 bp, Akkermansia muciniphila
atgcccggcggcaacctgccgacgctgcccgtcaagcgggtggtgcgtcccactccctccattccggaccatgaagttgtacgccagatagggagcggcgcgtacggagaagtatggctggcaaaatccctgaccggggcgtggcgcgccgtcaaaatcgtatggagggaggattttgaagacgagcgctctttcaaccgggaatttgagggcattctccagtatgaacccatcgcccgcaaccatccggggctggtccatatcctgcatgtagggaggcatgaccaggattccccgttttattattacgtcatggaactgggcgacgacgcccgcaccggagttcatattacaccggacgaatatattccgcgcacgctccagacggacaagaagttttccggcaacaagcctcttcccctggattactgcctggaggtaggcagccagctggcccacgccctgctgtacctgcacagcaagaacctgacgcaccgggacatcaagccggcgaacgtcatctttgtcaacgggcgccccaaactggcggacataggcctggtggcccatctggaccagcgcagctttgtagggacggagggattcatcccccccgacggccccggcacccggcgggcggacgtttacgcgctggccaaggttctgtatgaaatcagcacgggaaaggaccgcatggattttcccgaactcccggatgacttgccggaaggcaccgtgcgcaagaaatggcaggccttcaacaccatcatttgccaggcggcggaaccccgcattgaagaatgctccattgattccgcagaggagctggcggaaaaaatagacgccctccgggggtatgaagtgccttcccgtttccgtcttcagaagaaaaagaaacgccgcaaactcagacgggccctccaacttctggctgcagccgccgccggagccctgactgcctactggggggctttatggctcaacaacagccagcatccgccggaggaacctgcctcggatattcatccggatatccactcatccgctccggaagaagaatcccggaccggatacgtgctggtgaccagctccccggcgggagcgtccgtgtatgatgcggacggcaactatctggatgaaactccctacggccccattgaactgccttccggctccccggtagcctataccatcaagaaatcggggtttgcggacaaggaagaggcgggaaccgtcaaaggagggtccacgctggccctgggcggcgtgctgaaagagtaccatccccctacggacagccagccctggaaggatacggagggtgttacgtacctgcccgcagaaacgcgccatgtggcgcaaggcccccttaccgccgccctgttcaacaaatttctgaaggaggaccgccagaaagggaacttccagatgaaaagggaacagacggaaccggggcatccggagaaggatgtggccctgctcacgcaggacggcatcacggcctacctggcgtggctgaacaagaaatgcgagcgggaggggctgctgggcaaggaattttccatcaatgcggatccgcttccgcaggcttccggcagcacggaaaaccacaatgcctacgtcctgaacgtcacccgcgtgttccaggtgcccattaccgtcaccaccaatccgccgggagccagcgtttttttcaataacaggctcatcgggcgtacccccattgaagaatacgtcaaccaggttccctacgtcattgaaatcaaactgccggggcacgccaccatgcgtcgcagggggctggatccgcaggacttatacctttccctgcagttggaaccggacaagtctgtcgtttttggctcgccctggaccaacagcctgggcatcaaactggtccctgtgggtgggaatgctctggtcatgacccacgaagtgcgcgtaaaggactttcaggaattcctgaaagctaccggaaggaaagctccggcccggcccggctttccccagggagaagaccacccggtggtgaatgtcagcaggcaggatgcgcgcgccttcgccagatggcttaccagcaaagagcgggccctgggcctgattgatcagcacgactcctaccgtcttcccaaggatgaggaatggagttcctgggtgcgtctgacggatgaacagggagcctccccctatgaaaagacgctgcctcatgaaaactcccgggaagccttcccgtgggggtattcatggccgccgcctgataaaacgggaaattttgcggaccagtccgccctgatttacctgccgtcctcccgcgttatcgtaggatataacgacggacagccgtatacggcccccgtaaaaacctttccgcccaaccacctgggcctgtacgacctggaaggaaacgtcatggaatgggtagacgattcctacggggggccggaatccctccccatccgcaactacggcgtcgcccgcggaggcagctacctgtccttccgccccaaacagctcaccacttccatccgcactcccctgccggaaaatacgagggataacgcgctgggcttccgtcttatcctgtcttccgaacgccccgccattccaacagctccctga

SEQ ID NO: 39 - DNA, 1611 bp, Akkermansia muciniphila
atgctgacgatcaaaaatctcacaaaatcccacgccggacggaccttgttcagggaaacggaaatgaccattaactggggggaacgggtggctctggttggccccaacggagcaggcaaatccaccctgttccgcatgattctgggagaagacacgccggacgaaggctccatcagcatggatgaatacgccatcgtgggctatcttccccaggaagccagcgaaccgaaggatgaaaccgtcctggaaatcgccctgggcatcacgccggaaatggaacaggccatccacaccatccggacggcggaaaacgccaacaaaacggatacgccggaatacgcggaagccattgacaccttcaacgccgccaacggttaccagctggagcccaaagccaagaaaattctcaaagggctggcctttcgggaaagcgacttccaccgccccgcccgggaaatgtccggcggctggattatgcgcgcgtacctggccaagctccttgtcctggagccggacctcctgatgctggacgaacctactaaccacctggacctcctgtccctgctgtggctccagcgatacctgaaaaactaccccggagccatcctgatgatttcccacgaccgggatttcatggatgagctggtggaaagcgtgtacgacatcgacaacgaagaactggtggaataccgcggcaattactcggacttcctccaacaaaaggacgtgcgcttcgagcagcttcaggcggcctaccgcaaccagcagaaggaaatagcgcacattcaggaatttattgaccgtttccgctccatcaattccaaagccgggcaagtccagagccgcatcaagcagctggaaaagatgaaaatcattcaaaaaccggtagcctgcaggaaagtatttaaattcaacttcccccagcctccgcgcagcacccagaaagtcattgagctggaaaaagtctgccaatcctatggcgaccgcagggtttatgaaaatttggacctgctggtggaacgcggggagcgcactgttcttgtaggcccgaacggcgcgggcaaatccactcttctcaaaatcctggcgggcatcatccccattgactccggacaacgcactcccggtaccacgacgcgcatcggctacttctcccaggcgcgaacggaaaacctgaacccggaaaataccgtgctggaggaaatcatgaaatgcagcgctgaaatccgggaggaagaagcgcgttccatcctgggttccttcctgttccggaggctggatgtggaaaaacgcgtcagcgttctttccggcggggaaaaatcgcggctcagcctggtcaaattcctggtggatccgcccaacctcctgctgatggacgagccgaccacccacctggaccttttgtccgtagaagccctggtgcaggctctgaagcattatgaaggaacactggtcttcatctcccacgatgtgcacttcatccgttccctggcacaaaaaaccctgcatgtgaaccgggggaccatcaccgcctacgcaggcggatatgactactatctggaaaagtcaggcattctggacgatgaaaaaggcggcatcacggcggaataa

SEQ ID NO: 40 - DNA, 444 bp, Akkermansia muciniphila
atgattcaaacgtatcaagtactccctgtggtggccatcgtatgctccgcttccgcctttgcccagaacgctgccgatcccgtgcagatggtcaagcagaatatcgacctgatttcttccgccaacaaggttttggacgacgtgaaggacaacgctgcggttgaaatcgccattaagcagctcaatgcgttgacccagcaggccaagcagctggacaagtccatggaaaagatgaggcttacttccgagcaggctatccgcatcaccaaattgaacggagacgcccaggacaccatcgtggatatgctggaaaattgcgagcgcattcaaaaggacaagctgatgactccggctttgctcaaggcggtgaatgattttgccgacgccgccaacatcgacgtggtggaaacgattacgaccgtggagcaaattgtggaagattga

SEQ ID NO: 41 - DNA, 948 bp, Akkermansia muciniphila
atgagcaatatcaacccattcattctaacagggatgatgccgctttcagcctcatccatgaaccgtgtctcctacatgtgcccggtcaccatcagcaatgatgtagtgcagggccagacggacattcaggattcccttaccgttgattccggcggaaatctttacatcatcaacgctcctgtttacgtgggcggccccaaccagccggaccacgggcaccgcaccgcccacctcgtcatccggaacggaggcgccatgacgctcctgggcaatctgccggaccatatgaccgttttcctgggggacaaagccaacggcagcctggaaatcaacggcggccgccttctgatgggccaggggcgcattcagggcgccagggagcatgaaggcagaatcgccatgacggacggctggctcttcgcctcggaagtggatctgccggcggagggctcggaactcgtgatcaggcacggcctgatgcgtatcagaaaactctccggcaatgcatccacccgcatttacggaggcgttctgcacgtaaaggaggaagcccgcgccagccgcatccatctgatagacgacggcgtgctgctgctgggcagcgtcaccagccagccttccgcggacgtcatggccggagcgggcatcaacttccgcggggacggcggagcgctggtaatccgcatcccccacccggaaaacgctctgacgcgcacgcgggaagcggaacatgtctttgacgaactgctccggaggggcaagctctttcatgacagtgaacccatgaccagcttccaggggttccatatgagggagttcacggggcatgacggactggcgtacgccgcgctgcgcccctccgcccagctgaacgcggaacagaatcaggttacccgcctgctccatacgttcatgtacggcggcagtgaaaaggacatgcccatctga

SEQ ID NO: 42 - DNA, 522 bp, Akkermansia muciniphila
atggataaacaatccacagatcataaagaggaaactctggtggccatgctggcatctttccgcaaggaagcctgttaccatgacaccttcgaggaagatttcctccgcaattttcatctcagaaaggaaaccgatcaggctgcccactctgcttggaaattgctgctcgaacgcctggacaattatctgcagaactttcgtggttggcagtgggtctatgcttccatgtccatcgtgacattggctgcggtaggcgttattatcgcatccggaaacatggatgaaccttctgaatcttacgtatcctccaccaaggataaggaagaaatactcctgacgaaaaaagccgttcccgtaagtaaggaaactattgaacgaacctcaaccgaagttgctcccacggaaaaacctgaattcaccacgggagactcttcatatgaaacatcggccaaagacaaccagctgaaacctgattcccatgccgataaaaaaccggtatcccgcgttctcattgagatgtaa

SEQ ID NO: 43 - DNA, 603 bp, Akkermansia muciniphila
atgacgtttgggagtctctcacagagtgcccttcctggcggtttcattccttacggcggtaatttttatgcttccaattacacgatctccctctggctggatacctcttccttaacggaaggaacccagaccacgctgtttgggtattatggcaccaatgcgggccaaagttacgggacaaatgccttgtatctgacgacagatgccaagcttggcatgggagatggaaatttggatacttctaccggctctttttcccaaaaccgtggagacgtttctgaaactcccgttgttttggagggaggtcttcttaacgtgactctagccgttactggcgcagaccaaagccagtctgtggaggtctatgtgaatggttccttgcttgacacgttgtcctacaacggcaacatgaacggaaatcgcactgatatccaaggatggattaatcccaatcttacatggggtgaaattcagtggacggatacaaaactttccgcggaacagattgccggttttgccggccttcaggttccggaaccggcctcggcttctctgggaatcctgggcctggccgttctgatgatgcgccgccgccgttcctga

SEQ ID NO: 44 - DNA, 330 bp, Akkermansia muciniphila
atgaaaaaattgatctatatgatagcggcagcggccgttgcgattccggtggtggccctggcccagggagcctgcggcagcggctcctgctccaagggagacaaggacatggctgaagccaaagagcacatgaaagagggcgccaaggctgccaaggacgccgcctccgaaaaaatgaaggaaggcaggcaggctgccagggacgcctatgaaaagggcaaggaaaccgccagggatgcttatcaggacagcagggacgccgttgaccatgcggcggacaggactgccgataaggccgaagccgtcggtgacgctgtgaaaaacggttaa

SEQ ID NO: 45 - DNA, 1458 bp, Akkermansia muciniphila
atgattccgctccgcattgttcttgcctccctggcatgcctgtacccgttctctctggctcaggagcctaaatcggatcccgataaaacgctgattatcatttctaccagcgatatccacggcaatctggacaatttcccaagactggccacactggtaaagcaataccgcgctaaatatccgcacgtgctgctggtggattcaggtgattatttcataggcaatccctatgtggacgactgtgaaaaacggggcgaaccccttactatcctgatgaacaagctggggtatgatgtagtgaccatcggaaaccatgatctggattacgggcaggaggccctgcgcgaccatatcaagggaatgccctccaccaagtttgtcattaccaacgccagcctttccccaactctggaaaactgtttttctccgtatgtcagcatcccgattaaaggaacgtccatttccgtaggggtcataggactggcagaccttcaaaccacggatgtgaggaggatgaccggcatctcatggaagctgccggatgaagaagactacaagggaatcacggacaggttccggctccaccataataccatcaacgtcatcctcagccatctgggatacggcaatgatctgaaaatgatgaagtattctccgaatatcgacgtcattcttggaggccatacccatgtcatgctgcccagcggtcatctcagaaccggaaccctgctcagccacacgggacacagcctgagccatgtaggcgttacggaaattattttctccacggaacatcccgtctccatcctttccaaatcaaccagggccgtttctttgaatgaggaaattcccgatgacccggaagtaaaggaaattgtccgccgattttccggaaatccgcttttcaaccagcaagtgggcgtcgccggagaagaaatcacgcacgtcaccataggcacccttttctgcaaggccattcagcaggcctcccattcggatattgccatttacaaccgcggcggagtacggtccaaaaaccatcttaacaaaggacccgttaccatcagggacatttacgagctggaacccttccgggaaaagatcgtcacctgctccatgagtaaagcggacattgaacaactgatcctgtccaaattcatgtctccgaccgatgacgaaggaggcgttctggaagtgtactgctccggattctcctaccagatcatggacggtgttacgcccagcattaccagcaccttgaaaaacggggtcatttacactgtcgcgatgggagactacctgtgcagcaatttcatattcccccaacgggggaacggcaaaccgacgggaatagatgtccgcaaagccctgattgattacctgaaacaaatcaaggagctgctcaatcctccgccgtccaagctacctatcatcaaagatacgacgttcgccctgtga

SEQ ID NO: 46 - DNA, 789 bp, Akkermansia muciniphila
atgaagaaatccttgttgtctttagctttaatctcaagtaccttgcttgccgtagaggcggcaacggtgcaaattgatttcggacgcagtgacgccacgacggacggcgtgctcaatatgaattatgatagtgcctccgccgctttgggcagcatgccgggaagcgtttctttggcatggagtacggcagaatggcctgtaggggataatggccataccaccaccaagacagttgaggaagaagccgattggaaaaatcctttcaacggcagcatgcctttcagcttgggggacacttttcgtgacggtcttttaacgcagacggccgacgggtccggctctttcactgtaacgttcagcggtcttgccgccggggagtattccttgtccatctttggaggtttcacaggcaaggatgcatttgccggtcaaacctggacgatcggaaacgccgatgcttccaatgccgtctggacaagcttcggcacagacgccagcgggaactgggccgaaatttcttccgtgacgggcgataattccggagtccttactccggcgaacgcttccacttccagcgctactgctaataaagggctttatgctacggtagagaatgtcgtggtaggggaagacgggacgcttacccttacgattcagggggatgggagcaaggggtacggccttacagcccttaattacctttccctgacgcaggtgccggaacccgctacggcagcattgagcctgctgggcgctgctgccctgttcctgcgccgccgcagggactga

SEQ ID NO: 47 - DNA, 1190 bp, Artificial Sequence
  transposon insert from pSAM_Akk
taacaggttggatgataagtccccggtcttcgtatgccgtcttctgcttggcgcgccctcgagcaattgcgctcgtaagaggttccaactttcaccataatgaaataagatcactaccgggcgtattttttgagttatcgagattttcaggagctaaggaagctaaaatggagaaaaaaatcactggatataccaccgttgatatatcccaatggcatcgtaaagaacattttgaggcatttcagtcagttgctcaatgtacctataaccagaccgttcagctggatattacggcctttttaaagaccgtaaagaaaaataagcacaagttttatccggcctttattcacattcttgcccgcctgatgaatgctcatccggaattccgtatggcaatgaaagacggtgagctggtgatatgggatagtgttcacccttgttacaccgttttccatgagcaaactgaaacgttttcatcgctctggagtgaataccacgacgatttccggcagtttctacacatatattcgcaagatgtggcgtgttacggtgaaaacctggcctatttccctaaagggtttattgagaatatgtttttcgtctcagccaatccctgggtgagtttcaccagttttgatttaaacgtggccaatatggacaacttcttcgcccccgttttcaccatgggcaaatattatacgcaaggcgacaaggtgctgatgccgctggcgattcaggttcatcatgccgtttgtgatggcttccatgtcggcagaatgcttaatgaattacaacagtactgcgatgagtggcagggcggggcgtaatttttttaaggcagttattggtgcccttaaacgcctggtgctacgcctgaataagtatgcgagagtagggaactgccaggcatcaaataaaacgaaaggctcagtcgaaagactgggcctttcgttttatctgttgtttgtcggtgaacgctctcctgagtaggacaaatccgccgggagcggatttgaacgttgcgaagcaacggcccggagggtggcgggcaggacgcccgccataaactgccaggcatcaaattaagcagaaggccatcctgacggatggcctttttgcgtttctacctgcagggcgcgccaagcagaagacggcatacgaagaccggggacttatcatccaacctgtta